European Patent Specification EP 4 060 034 B1, published October 2, 2024. Title: Novel hydrolase variant and a method for producing L-tryptophan using the same. Applicant: CJ CheilJedang Corporation. The sequence listing filed with the application follows.

SEQUENCE LISTING (10 sequences)

SEQ ID NO: 1 - protein, 585 aa, Artificial Sequence
  ynbC
MENSRIPGEHFFTTSDNTALFYRHWPALQPGAKKVIVLFHRGHEHSGRLQHLVDELAMPDTAFYAWDARGHGKSSGPRGYSPSLARSVRDVDEFVRFAASDSQVGLEEVVVIAQSVGAVLVATWIHDYAPAIRGLVLASPAFKVKLYVLLARPALALWHRLRGLFFINSYVKGRYLTHDRQRGASFNNDPLITRAIAVNILLDLYKTSERIIRDAAAITLPTQLLISGDDYVVHRQPQIDFYQRLRSPLKELHLLPGFYHDTLGEENRALAFEKMQSFISRLYANKSQKFDYQHEDCTGPSADRWRLLSGGPVPLSPVDLAYRFMRKAMKLFGTHSSGLHLGMSTGFDSGSSLDYVYQNQPQGSNAFGRLVDKIYLNSVGWRGIRQRKTHLQILIKQAVADLHAKGLAVRVVDIAAGHGRYVLDALANEPAVSDILLRDYSELNVAQGQEMIAQRGMSGRVRFEQGDAFNPEELSALTPRPTLAIVSGLYELFPENEQVKNSLAGLANAIEPGGILIYTGQPWHPQLEMIAGVLTSHKDGKPWVMRVRSQGEMDSLVRDAGFDKCTQRIDEWGIFTVSMAVRRDN

SEQ ID NO: 2 - DNA, 1758 bp, Artificial Sequence
  ynbC
atggaaaattcacgcatccctggggaacatttttttaccaccagtgataatacagcgttgttttatcggcactggcccgctttacagcccggggcgaaaaaggtcatcgtcttatttcatcgcgggcatgaacattctggtcgtctacaacatctcgttgatgaactggcgatgccagatactgctttttatgcctgggatgcccgagggcatggaaaaagttcggggccgcgtggttatagcccatctcttgcgcgttcagtgcgggatgtcgatgaatttgtccgttttgctgccagcgacagccaggttggactggaagaggtggtagtgatcgcgcaaagcgtcggcgcagtgctggttgccacatggattcatgattatgcacctgcaattcgcgggctggtgctggcttctccggcctttaaggttaaattgtatgtgctgctggcacgtcctgcgctggcgttatggcatcgtctgcgtggtctgttttttattaattcctatgtgaaaggacgctatttgacccacgatcggcaacggggggcgagtttcaataatgatccgctgatcacacgggcgattgccgttaatatcttgctcgatctctacaaaacgtctgaacgtattattagagatgcggcggcgattacgctccccacgcaacttctgatatcaggcgatgactatgtggtgcatcgccaaccgcagattgatttttatcagagattacgtagccctctgaaagagctgcatctgctgccaggcttttatcacgacacgttgggtgaagagaacagggcgctggcatttgaaaaaatgcaaagctttattagtcgtttatatgctaacaaatcgcaaaaatttgattatcagcatgaagactgcacaggaccatcagcggatcgatggcggctactttctggtggacccgtgccattatcgccggttgatttagcgtatcgctttatgcgaaaggcgatgaaattgttcgggacgcactcttcgggcctgcatctcggaatgagcaccggctttgattcaggcagttcgctggattatgtctatcaaaatcaaccgcaaggtagtaacgcattcgggcgtttagtcgacaaaatctacctgaacagtgttggctggcgcggtattcgccagcgcaaaacccatttacaaatactgattaaacaagccgttgccgatctccacgccaaaggtttagccgtccgcgtggttgacattgccgcagggcatgggcgctatgtactggatgcgctggcaaacgagcctgccgtaagcgatattttgttacgtgattacagcgagttaaatgttgcacaggggcaagagatgattgctcaacggggaatgtctgggcgggtgcgttttgaacagggcgatgcgtttaacccggaggaactcagcgcgttaactccgcggcctacgctggcgattgtctctggcctgtatgagctttttcccgaaaatgagcaggtaaaaaactcactcgcaggtcttgccaatgccatcgaaccgggcggcattctcatctacaccgggcagccgtggcaccctcaactggagatgattgccggggtgttaaccagtcataaagatggtaaaccgtgggtaatgcgcgtgcgttcgcaaggggagatggattcactcgtgcgtgatgccggatttgataaatgcacacaacggattgatgagtggggtatttttacggtttcgatggcggtgcgtcgtgataactga

SEQ ID NO: 3 - protein, 585 aa, Unknown
  ynbC
MENSRIPGEHFFTTSDNTALFYRHWPALQPGAKKVIVLFHRGHEHSGRLQHLVDELAMPDTAFYAWDARGHGKSSGPRGYSPSLARSVRDVDEFVRFAASDSQVGLEEVVVIAQSVGAVLVATWIHDYAPAIRGLVLASPAFKVKLYVPLARPALALWHRLRGLFFINSYVKGRYLTHDRQRGASFNNDPLITRAIAVNILLDLYKTSERIIRDAAAITLPTQLLISGDDYVVHRQPQIDFYQRLRSPLKELHLLPGFYHDTLGEENRALAFEKMQSFISRLYANKSQKFDYQHEDCTGPSADRWRLLSGGPVPLSPVDLAYRFMRKAMKLFGTHSSGLHLGMSTGFDSGSSLDYVYQNQPQGSNAFGRLVDKIYLNSVGWRGIRQRKTHLQILIKQAVADLHAKGLAVRVVDIAAGHGRYVLDALANEPAVSDILLRDYSELNVAQGQEMIAQRGMSGRVRFEQGDAFNPEELSALTPRPTLAIVSGLYELFPENEQVKNSLAGLANAIEPGGILIYTGQPWHPQLEMIAGVLTSHKDGKPWVMRVRSQGEMDSLVRDAGFDKCTQRIDEWGIFTVSMAVRRDN

SEQ ID NO: 4 - DNA, 1758 bp, Unknown
  ynbC
atggaaaattcacgcatccctggggaacatttttttaccaccagtgataatacagcgttgttttatcggcactggcccgctttacagcccggggcgaaaaaggtcatcgtcttatttcatcgcgggcatgaacattctggtcgtctacaacatctcgttgatgaactggcgatgccagatactgctttttatgcctgggatgcccgagggcatggaaaaagttcggggccgcgtggttatagcccatctcttgcgcgttcagtgcgggatgtcgatgaatttgtccgttttgctgccagcgacagccaggttggactggaagaggtggtagtgatcgcgcaaagcgtcggcgcagtgctggttgccacatggattcatgattatgcacctgcaattcgcgggctggtgctggcttctccggcctttaaggttaaattgtatgtgccgctggcacgtcctgcgctggcgttatggcatcgtctgcgtggtctgttttttattaattcctatgtgaaaggacgctatttgacccacgatcggcaacggggggcgagtttcaataatgatccgctgatcacacgggcgattgccgttaatatcttgctcgatctctacaaaacgtctgaacgtattattagagatgcggcggcgattacgctccccacgcaacttctgatatcaggcgatgactatgtggtgcatcgccaaccgcagattgatttttatcagagattacgtagccctctgaaagagctgcatctgctgccaggcttttatcacgacacgttgggtgaagagaacagggcgctggcatttgaaaaaatgcaaagctttattagtcgtttatatgctaacaaatcgcaaaaatttgattatcagcatgaagactgcacaggaccatcagcggatcgatggcggctactttctggtggacccgtgccattatcgccggttgatttagcgtatcgctttatgcgaaaggcgatgaaattgttcgggacgcactcttcgggcctgcatctcggaatgagcaccggctttgattcaggcagttcgctggattatgtctatcaaaatcaaccgcaaggtagtaacgcattcgggcgtttagtcgacaaaatctacctgaacagtgttggctggcgcggtattcgccagcgcaaaacccatttacaaatactgattaaacaagccgttgccgatctccacgccaaaggtttagccgtccgcgtggttgacattgccgcagggcatgggcgctatgtactggatgcgctggcaaacgagcctgccgtaagcgatattttgttacgtgattacagcgagttaaatgttgcacaggggcaagagatgattgctcaacggggaatgtctgggcgggtgcgttttgaacagggcgatgcgtttaacccggaggaactcagcgcgttaactccgcggcctacgctggcgattgtctctggcctgtatgagctttttcccgaaaatgagcaggtaaaaaactcactcgcaggtcttgccaatgccatcgaaccgggcggcattctcatctacaccgggcagccgtggcaccctcaactggagatgattgccggggtgttaaccagtcataaagatggtaaaccgtgggtaatgcgcgtgcgttcgcaaggggagatggattcactcgtgcgtgatgccggatttgataaatgcacacaacggattgatgagtggggtatttttacggtttcgatggcggtgcgtcgtgataactga

SEQ ID NO: 5 - DNA, 40 bp, Artificial Sequence
  Forward Primer
ggaattcgagctcggtacccatggaaaattcacgcatccc

SEQ ID NO: 6 - DNA, 21 bp, Artificial Sequence
  Reverse Primer
acgtgccagcagcacatacaa

SEQ ID NO: 7 - DNA, 21 bp, Artificial Sequence
  Forward Primer
ttgtatgtgctgctggcacgt

SEQ ID NO: 8 - DNA, 40 bp, Artificial Sequence
  Reverse Primer
gttatccctagcggatccccgcaggcccgaagagtgcgtc

SEQ ID NO: 9 - DNA, 20 bp, Artificial Sequence
  Forward Primer
ggcggactccttgacaggat

SEQ ID NO: 10 - DNA, 20 bp, Artificial Sequence
  Reverse Primer
ccagcgaactgcctgaatca